European Patent Application EP 4 393 945 A1, published July 3, 2024. Title: 抗RSV病毒抗体及其应用. Applicant: 甘李药业股份有限公司. Application CN. The sequence listing filed with the application follows.

SEQUENCE LISTING (124 sequences)

SEQ ID NO: 1 - protein, 125 aa, synthetic construct
EVKLEESGPELVKPGASVKISCKTSGYAFSDSWMNWVKQRPGQGLEWIGRIYPGDGDTQYNGKVKGKATLTADKSSSTAYMQVSSLTSVDSAVYFCAREGGMITSSGYYHALDYWGQGTSVTVSS

SEQ ID NO: 2 - protein, 110 aa, synthetic construct
DIVMTQSPASLAVSLGQRTTISCRASESVDSYGNSFLNWYQQKPGQPPKVLIYLASNLESGVPARFSGSGSRTDFTLIIDPVEADDAATYYCQQNNEDPTFGGGTKLEIK

SEQ ID NO: 3 - protein, 116 aa, synthetic construct
QVQLEESGAELVRSGASVKLSCTASGFNIKDYYIHWVKQRPEQGLEWIGWNDPENGDTEYAPKFQGKATMTADTSSNTVYLQLSSLTSEDSAVYFCKSFDSYLEYWGQGTSVTVSS

SEQ ID NO: 4 - protein, 112 aa, synthetic construct
DIVMTQTTLSLPVNLGDQASISCRSSQSLVHTDGNTFLEWYLQRPGQSPKLLIYKVSIRFSGVPDRFSGSGSGTDFTLKISRVETEDLGVYYCFQGSHVPRTFGGGTKLEIK

SEQ ID NO: 5 - protein, 121 aa, synthetic construct
EVQLEESGPELVKPGASVKISCKSSAQTFSGSWINWVKQRPGQGLEWIGRIFPGDGDTKYNMNFTGKATLTADKSSNTAYMHVSSLTSVDSAVYFCARYDGYYDIGYFDVWGAGTTVTVSS

SEQ ID NO: 6 - protein, 111 aa, synthetic construct
DIVMTQTPASLAVSLGQRATISCRASASVDSYGNKFIHWYQQKPGQPPKLLISLASNLESGVPARFSGSGSRTDFTLTIDPVEADDAATYYCQQTNEDPWTFGGGTKLEIK

SEQ ID NO: 7 - protein, 121 aa, synthetic construct
EVQLEESGAELVRSGASVKLSCTASGFNIKDYYMHWVKQRPEQGLEWIGWIDPENGDTEYAPKFQGKATLTADTSSNTAYLQLSTLTSEDNAVYYCNAAYYGDYVEDMDYWGQGTSVTVSS

SEQ ID NO: 8 - protein, 112 aa, synthetic construct
DIVMTQTPLSLSVSLGDQASISCRSSQSIVHSDGNTFLEWYLQKPGQSPKLLIYKVSNRFSGVPDRFSGSGSGTDFTLKISRVEAEDLGVYYCFQASHLPRTFGGGTKLEIK

SEQ ID NO: 9 - protein, 122 aa, synthetic construct
QVKLEESGPGILQPSQTLSLTCSFSGFSLSTSGMGVSWIRQPSGKGLEWLAHIYWDDDKNYNPSLKSRLTISKDTSRNQVFLKITSVDTADTATYYCARKIYYDYDYALDYWGQGTSVTVSS

SEQ ID NO: 10 - protein, 111 aa, synthetic construct
DIVMTQAAFSNPVTLGTSASISCRSSKSLLHSNGITYLCWFLQKPGQSPQLLIYQMSNLASGVPDRFSGSGSGTDFTLRISRVEAEDVGVYYCAQNLELWTFGGGTKLEIK

SEQ ID NO: 11 - protein, 119 aa, synthetic construct
EVKLLESGGGLVQPGGSLKLSCAASGFDFSRYWMSWVRQAPGKGLEWIGEINPDSSTINYTPSLKDKFIISRDNAKNTLYLQMSKVRSEDTALYYCARRGGISYAMDYWGQGTSVTVSS

SEQ ID NO: 12 - protein, 112 aa, synthetic construct
DIVITQDELSNPVTSGESVSISCRSSKSLLYKDGKTYLNWFLQRPGQSPQLLIYLMSTRASGVSDRFSGSGSGTDFTLEISRVKAEDVGVYYCQQLVEYPRTFGGGTKLEIK

SEQ ID NO: 13 - protein, 122 aa, synthetic construct
EVKLQESGPGMLQPSQTLSLTCSFSGFSLSTSGMGVSWIRQPSGKGLEWLAHIYWDDDKNFNPSLRSRLIISKDPSRNQVFLEITSVDTADTATYFCARKLYNDYDYILDYWGQGTSVTVSS

SEQ ID NO: 14 - protein, 111 aa, synthetic construct; identical to SEQ ID NO: 10

SEQ ID NO: 15 - protein, 125 aa, synthetic construct
QVKLEESGPELVKPGASVKISCKASGYAFSSSWVNWVQQRPGQGLEWIGRIYPGDGETKYSGKFRGKATLTADKSSNTVYMQVSSLTSVDSAVYFCAREGGLITSSGYYHAMDYWGQGTSVTVSS

SEQ ID NO: 16 - protein, 110 aa, synthetic construct
DIVLTQSPPSLAVSLGQRATISCRASKSVDSYGNGFMHWYQQKPGQPPKLLIFLASNLESGVPARFSGSGSRTDFTLTIDPVEADDAASYYCQQSDEDPTFGGGTKLEIK

SEQ ID NO: 17 - protein, 125 aa, synthetic construct
QVQLEESGPELVKPGASVKISCKASGYAFSSSWMNWVKQRPGQGLEWIGRIYPGDGDTQYHGKVKGKATLTADKSSSTAYMQVSSLTSVDSAVYFCAREGGMITSNGYYHALDYWGQGTSVTVSS

SEQ ID NO: 18 - protein, 110 aa, synthetic construct
DIVMTQTTASLAVSQGQRATISCSASESVDSYGNSFMNWYQQKPGQPPKVLIYLASNLESGVPARFSGSGSRTDFTLTIDPVEADDAATYYCQQNNEDPTFGGGTKLEIK

SEQ ID NO: 19 - protein, 122 aa, synthetic construct
QVTLKESGPALVKPTQTLTLTCTFSGFSLSTSGMGVSWIRQPPGKALEWLAHIYWDDDKNFNPSLRSRLTITKDTSKNQVVLTMTNMDPVDTATYYCARKLYNDYDYILDYWGQGTTVTVSS

SEQ ID NO: 20 - protein, 111 aa, synthetic construct
DIVMTQSPLSLPVTPGEPASISCRSSKSLLHSNGITYLCWYLQKPGQSPQLLIYQMSNLASGVPDRFSGSGSGTDFTLKISRVEAEDVGVYYCAQNLELWTFGQGTRLEIK

SEQ ID NO: 21 - protein, 122 aa, synthetic construct
QVTLKESGPALVKPTQTLTLTCTFSGFSLSTSGMGVSWIRQPPGKALEWLAHIYWDDDKNFNPSLRSRLTITKDPSKNQVVLTMTNMDPVDTATYFCARKLYNDYDYILDYWGQGTTVTVSS

SEQ ID NO: 22 - protein, 111 aa, synthetic construct
DIVMTQSPLSLPVTPGEPASISCRSSKSLLHSNGITYLCWFLQKPGQSPQLLIYQMSNLASGVPDRFSGSGSGTDFTLKISRVEAEDVGVYYCAQNLELWTFGQGTRLEIK

SEQ ID NO: 23 - protein, 122 aa, synthetic construct
QVTLRESGPALVKPTQTLTLTCTFSGFSLSTSGMGVSWIRQPPGKALEWLAHIYWDDDKNFNPSLRSRLTISKDPSKNQVVLTMTNMDPVDTATYFCARKLYNDYDYILDYWGQGSLVTVSS

SEQ ID NO: 24 - protein, 112 aa, synthetic construct
DIVMTQSPDSLSVSLGERATINCRSSKSLLHSNGITYLCWFQQKPGQPPKLLIYQMSNLASGVPDRFSGSGSGTDFTLTISSLQAEDVAVYYCAQNLELWTFGGGTKVEIKR

SEQ ID NO: 25 - protein, 122 aa, synthetic construct
QVTLRESGPALVKPTQTLTLTCTVSGFSLSTSGMGVSWIRQPPGKALEWLAHIYWDDDKNFNPSLRSRLTISKDTSKNQVVLTMTNMDPVDTATYYCARKLYNDYDYILDYWGQGSLVTVSS

SEQ ID NO: 26 - protein, 112 aa, synthetic construct
DIVMTQSPDSLSVSLGERATINCRSSKSLLHSNGITYLCWYQQKPGQPPKLLIYQMSNLASGVPDRFSGSGSGTDFTLTISSLQAEDVAVYYCAQNLELWTFGGGTKVEIKR

SEQ ID NO: 27 - protein, 122 aa, synthetic construct
QVQLQESGPGLVKPSETLSLTCTFSGFSLSTSGMGVSWIRQHPGKGLEWLAHIYWDDDKNFNPSLRSRLTISKDPSKNQVSLKLSSVTAADTAVYFCARKLYNDYDYILDYWGQGTTVTVSS

SEQ ID NO: 28 - protein, 111 aa, synthetic construct
DIQMTQSPSSLSASVGDRVTITCRSSKSLLHSNGITYLCWFQQKPGKAPKLLIYQMSNLASGVPSRFSGSGSGTDFTLTISSLQPEDFATYYCAQNLELWTFGQGTKVEIK

SEQ ID NO: 29 - protein, 133 aa, synthetic construct
MDMRVPAQLLGLLLLWLSGARCDIVMTQSPLSLPVTPGEPASISCRSSKSLLHSNGITYLGWFLQKPGQSPQLLIYQMSNLASGVPDRFSGSGSGTDFTLKISRVEAEDVGVYYCAQNLELWTFGQGTRLEIK

SEQ ID NO: 30 - protein, 133 aa, synthetic construct
MDMRVPAQLLGLLLLWLSGARCDIVMTQSPLSLPVTPGEPASISCRSSKSLLHSNGITYLIWFLQKPGQSPQLLIYQMSNLASGVPDRFSGSGSGTDFTLKISRVEAEDVGVYYCAQNLELWTFGQGTRLEIK

SEQ ID NO: 31 - protein, 133 aa, synthetic construct
MDMRVPAQLLGLLLLWLSGARCDIVMTQSPLSLPVTPGEPASISCRSSKSLLHSNGITYLAWFLQKPGQSPQLLIYQMSNLASGVPDRFSGSGSGTDFTLKISRVEAEDVGVYYCAQNLELWTFGQGTRLEIK

SEQ ID NO: 32 - protein, 133 aa, synthetic construct
MDMRVPAQLLGLLLLWLSGARCDIVMTQSPLSLPVTPGEPASISCRSSKSLLHSNGITYLMWFLQKPGQSPQLLIYQMSNLASGVPDRFSGSGSGTDFTLKISRVEAEDVGVYYCAQNLELWTFGQGTRLEIK

SEQ ID NO: 33 - protein, 133 aa, synthetic construct
MDMRVPAQLLGLLLLWLSGARCDIVMTQSPLSLPVTPGEPASISCRSSKSLLHSNGITYLQWFLQKPGQSPQLLIYQMSNLASGVPDRFSGSGSGTDFTLKISRVEAEDVGVYYCAQNLELWTFGQGTRLEIK

SEQ ID NO: 34 - protein, 133 aa, synthetic construct
MDMRVPAQLLGLLLLWLSGARCDIVMTQSPLSLPVTPGEPASISCRSSKSLLHSNGITYLNWFLQKPGQSPQLLIYQMSNLASGVPDRFSGSGSGTDFTLKISRVEAEDVGVYYCAQNLELWTFGQGTRLEIK

SEQ ID NO: 35 - protein, 133 aa, synthetic construct
MDMRVPAQLLGLLLLWLSGARCDIVMTQSPLSLPVTPGEPASISCRSSKSLLHSNGITYLVWFLQKPGQSPQLLIYQMSNLASGVPDRFSGSGSGTDFTLKISRVEAEDVGVYYCAQNLELWTFGQGTRLEIK

SEQ ID NO: 36 - protein, 133 aa, synthetic construct
MDMRVPAQLLGLLLLWLSGARCDIVMTQSPLSLPVTPGEPASISCRSSKSLLHSNGITYLPWFLQKPGQSPQLLIYQMSNLASGVPDRFSGSGSGTDFTLKISRVEAEDVGVYYCAQNLELWTFGQGTRLEIK

SEQ ID NO: 37 - protein, 5 aa, synthetic construct
DSWMN

SEQ ID NO: 38 - protein, 17 aa, synthetic construct
RIYPGDGDTQYNGKVKG

SEQ ID NO: 39 - protein, 16 aa, synthetic construct
EGGMITSSGYYHALDY

SEQ ID NO: 40 - protein, 15 aa, synthetic construct
RASESVDSYGNSFLN

SEQ ID NO: 41 - protein, 7 aa, synthetic construct
LASNLES

SEQ ID NO: 42 - protein, 8 aa, synthetic construct
QQNNEDPT

SEQ ID NO: 43 - protein, 5 aa, synthetic construct
DYYIH

SEQ ID NO: 44 - protein, 17 aa, synthetic construct
WNDPENGDTEYAPKFQG

SEQ ID NO: 45 - protein, 7 aa, synthetic construct
FDSYLEY

SEQ ID NO: 46 - protein, 16 aa, synthetic construct
RSSQSLVHTDGNTFLE

SEQ ID NO: 47 - protein, 7 aa, synthetic construct
KVSIRFS

SEQ ID NO: 48 - protein, 9 aa, synthetic construct
FQGSHVPRT

SEQ ID NO: 49 - protein, 5 aa, synthetic construct
GSWIN

SEQ ID NO: 50 - protein, 17 aa, synthetic construct
RIFPGDGDTKYNMNFTG

SEQ ID NO: 51 - protein, 12 aa, synthetic construct
YDGYYDIGYFDV

SEQ ID NO: 52 - protein, 15 aa, synthetic construct
RASASVDSYGNKFIH

SEQ ID NO: 53 - protein, 7 aa, synthetic construct
LASNLES

SEQ ID NO: 54 - protein, 9 aa, synthetic construct
QQTNEDPWT

SEQ ID NO: 55 - protein, 5 aa, synthetic construct
DYYMH

SEQ ID NO: 56 - protein, 17 aa, synthetic construct
WIDPENGDTEYAPKFQG

SEQ ID NO: 57 - protein, 12 aa, synthetic construct
AYYGDYVEDMDY

SEQ ID NO: 58 - protein, 16 aa, synthetic construct
RSSQSIVHSDGNTFLE

SEQ ID NO: 59 - protein, 7 aa, synthetic construct
KVSNRFS

SEQ ID NO: 60 - protein, 9 aa, synthetic construct
FQASHLPRT

SEQ ID NO: 61 - protein, 7 aa, synthetic construct
TSGMGVS

SEQ ID NO: 62 - protein, 16 aa, synthetic construct
HIYWDDDKNYNPSLKS

SEQ ID NO: 63 - protein, 12 aa, synthetic construct
KIYYDYDYALDY

SEQ ID NO: 64 - protein, 16 aa, synthetic construct
RSSKSLLHSNGITYLC

SEQ ID NO: 65 - protein, 7 aa, synthetic construct
QMSNLAS

SEQ ID NO: 66 - protein, 8 aa, synthetic construct
AQNLELWT

SEQ ID NO: 67 - protein, 5 aa, synthetic construct
RYMWS

SEQ ID NO: 68 - protein, 17 aa, synthetic construct
EINPDSSTINYTPSLKD

SEQ ID NO: 69 - protein, 10 aa, synthetic construct
RGGISYAMDY

SEQ ID NO: 70 - protein, 16 aa, synthetic construct
RSSKSLLYKDGKTYLN

SEQ ID NO: 71 - protein, 7 aa, synthetic construct
LMSTRAS

SEQ ID NO: 72 - protein, 9 aa, synthetic construct
QQLVEYPRT

SEQ ID NO: 73 - protein, 7 aa, synthetic construct
TSGMGVS

SEQ ID NO: 74 - protein, 16 aa, synthetic construct
HIYWDDDKNFNPSLRS

SEQ ID NO: 75 - protein, 12 aa, synthetic construct
KLYNDYDYILDY

SEQ ID NO: 76 - protein, 16 aa, synthetic construct
RSSKSLLHSNGITYLC

SEQ ID NO: 77 - protein, 7 aa, synthetic construct
QMSNLAS

SEQ ID NO: 78 - protein, 8 aa, synthetic construct
AQNLELWT

SEQ ID NO: 79 - protein, 5 aa, synthetic construct
SSWVN

SEQ ID NO: 80 - protein, 17 aa, synthetic construct
RIYPGDGETKYSGKFRG

SEQ ID NO: 81 - protein, 16 aa, synthetic construct
EGGLITSSGYYHAMDY

SEQ ID NO: 82 - protein, 15 aa, synthetic construct
RASKSVDSYGNGFMH

SEQ ID NO: 83 - protein, 7 aa, synthetic construct
LASNLES

SEQ ID NO: 84 - protein, 8 aa, synthetic construct
QQSDEDPT

SEQ ID NO: 85 - protein, 5 aa, synthetic construct
SSWMN

SEQ ID NO: 86 - protein, 17 aa, synthetic construct
RIYPGDGDTQYHGKVKG

SEQ ID NO: 87 - protein, 16 aa, synthetic construct
EGGMITSNGYYHALDY

SEQ ID NO: 88 - protein, 14 aa, synthetic construct
SASESVDSYGNFMN

SEQ ID NO: 89 - protein, 7 aa, synthetic construct
LASNLES

SEQ ID NO: 90 - protein, 8 aa, synthetic construct
QQNNEDPT

SEQ ID NO: 91 - DNA, 375 bp, synthetic construct
  source 1..375: mol_type = other DNA
gaagtgaagctggaggagtctggacctgagctggtgaagcctggggcctcagtgaagatttcctgcaaaacttctggctacgcattcagtgactcttggatgaactgggtgaaacagaggcctggacagggtcttgaatggattggacggatttatcctggagatggagatactcagtataatgggaaggtcaagggcaaggccacactgactgcagacaaatcctccagcacagcctacatgcaggtcagcagcctgacctctgtggactctgcggtctatttctgtgcaagagagggaggcatgattacgtcgagtgggtattaccatgctttggactactggggtcaaggaacctcagtcaccgtctcctca

SEQ ID NO: 92 - DNA, 330 bp, synthetic construct
  source 1..330: mol_type = other DNA
gatattgtgatgacacagtctccagcttctttggctgtgtctctagggcagaggaccaccatatcctgtagagccagtgaaagtgttgatagttatggcaatagttttttgaactggtaccagcagaaaccaggacagccacccaaagtcctcatctatcttgcgtccaacctagaatctggggtccctgccaggttcagtggcagtgggtctaggacagacttcaccctcatcattgatcctgtggaggctgatgatgctgcaacctattactgtcaacaaaataatgaggatccgacgttcggtggaggcaccaagctggaaatcaaa

SEQ ID NO: 93 - DNA, 348 bp, synthetic construct
  source 1..348: mol_type = other DNA
caggttcagctggaggagtctggggcagagcttgtgaggtcaggggcctcagtcaagttgtcctgcacagcttctggcttcaacattaaagactactatatacactgggtgaagcagaggcctgaacagggcctggagtggattggatggaatgatcctgagaatggtgatacagagtatgccccgaagttccagggcaaggccactatgactgcagacacatcctccaacacagtctacctgcagctcagcagcctgacatctgaggacagtgccgtctatttctgtaagagttttgattcttatctggagtactggggtcaaggaacctcagtcaccgtctcctca

SEQ ID NO: 94 - DNA, 336 bp, synthetic construct
  source 1..336: mol_type = other DNA
gacattgtgatgacacagactacactctccctgcctgtcaatcttggagatcaagcctccatctcttgcagatctagtcagagccttgtacatactgatggaaacacctttttagaatggtacctgcagagaccaggccagtctccaaagctcctgatctacaaagtttccatccgattttctggggtcccagacaggttcagtggcagtggatcagggacagatttcacactcaagatcagcagagtggagactgaggatctgggagtttattactgctttcaaggttcacatgttcctcggacgttcggtggaggcaccaagctggaaatcaaa

SEQ ID NO: 95 - DNA, 363 bp, synthetic construct
  source 1..363: mol_type = other DNA
gaagtacagctggaggagtctggacctgagctggtgaagcctggggcctcagtgaagatttcgtgcaaatcttctgcccaaacattcagtggctcttggataaattgggtgaaacagaggcccggacagggtcttgagtggattggacggatttttcctggagatggagatactaaatacaatatgaacttcacgggcaaggccacactgactgcagacaaatcctccaatacagcctacatgcacgtcagtagcctgacctctgtggactctgcggtctatttctgtgcacgatatgatggttactacgatatcggctatttcgatgtctggggcgcagggaccacggtcaccgtctcttca

SEQ ID NO: 96 - DNA, 333 bp, synthetic construct
  source 1..333: mol_type = other DNA
gatattgtgatgacacagactccagcttctttggctgtgtctctagggcagagggccaccatatcctgcagagccagtgcaagtgttgatagttatggcaataaatttatacactggtaccaacagaaaccaggacagccacccaaactcctcatctctcttgcatccaacctagaatctggggtccctgccaggttcagtggcagtgggtctaggacagacttcaccctcaccattgatcctgtggaggctgatgatgctgcaacctattactgtcagcaaactaatgaggatccgtggacgttcggtggaggcaccaagctggaaatcaaa

SEQ ID NO: 97 - DNA, 363 bp, synthetic construct
  source 1..363: mol_type = other DNA
gaggtgcagctggaggagtcaggggcagagcttgtgaggtcaggggcctcagtcaagttgtcctgcacagcttctggcttcaacattaaagactactatatgcactgggtgaaacagaggcctgaacagggcctggagtggattggatggattgatcctgagaatggtgatactgaatatgccccgaagttccagggcaaggccactttgactgcagacacatcctccaacacagcctacctgcagctcagcaccctgacatctgaggacaatgccgtctattactgtaatgcagcctactatggtgactacgtggaagatatggactactggggtcaaggaacctcagtcaccgtctcctca

SEQ ID NO: 98 - DNA, 336 bp, synthetic construct
  source 1..336: mol_type = other DNA
gacattgtgatgacacagactccactctccctgtctgtcagtcttggagatcaagcctccatctcttgcagatctagtcagagcattgtacatagtgatggaaacacctttttagaatggtacctgcagaaaccaggccagtctcctaagctcctgatctacaaagtttccaaccgattttctggggtcccagacaggttcagtggcagtggatcagggacagatttcacactcaagatcagcagagtggaggctgaggatctgggagtttattactgctttcaagcttcacatcttcctcggacgttcggtggaggcaccaagctggaaatcaaa

SEQ ID NO: 99 - DNA, 366 bp, synthetic construct
  source 1..366: mol_type = other DNA
caagttaagctggaggagtcaggccctgggatattgcagccctcccagaccctcagtctgacttgttctttctctgggttttcattgagcacttctggtatgggtgtgagctggattcgtcagccttcaggaaagggtctggagtggctggcccacatttactgggatgatgacaagaactataacccatccctgaagagccgactcacaatctccaaggatacctccagaaatcaggtattcctcaagatcaccagtgtggacactgcagatactgccacatactactgtgctcgaaagatctactatgattacgactatgctttggactactggggtcaaggaacctcagtcaccgtctcctca

SEQ ID NO: 100 - DNA, 333 bp, synthetic construct
  source 1..333: mol_type = other DNA
gatattgtgatgacgcaggctgccttctccaatccagtcactcttggaacatcagcttccatctcctgcaggtctagtaagagtctcctacatagtaatggcatcacttatttgtgttggtttctgcagaagccaggccagtctcctcagctcctgatttatcagatgtccaaccttgcctcaggagtcccagacaggttcagtggcagtgggtcaggaactgatttcacactgagaatcagcagagtggaggctgaggatgtgggtgtttattactgtgctcaaaatctagagctgtggacgttcggtggaggcaccaagctggaaatcaaa

SEQ ID NO: 101 - DNA, 357 bp, synthetic construct
  source 1..357: mol_type = other DNA
gaggtgaagcttctcgagtctggaggtggcctggtgcagcctggaggatccctgaaactctcctgtgcagcctcaggattcgattttagtagatactggatgagttgggtccggcaggctccagggaaagggctagaatggattggagaaattaatccagatagcagtacgataaactatacgccatctctaaaggataaattcatcatctccagagacaacgccaaaaatacgctgtacctgcaaatgagcaaagtgagatctgaggacacagccctttattactgtgcaagaaggggagggatttcctatgctatggactactggggtcaaggaacctcagtcaccgtctcctca

SEQ ID NO: 102 - DNA, 336 bp, synthetic construct
  source 1..336: mol_type = other DNA
gatattgtgataacccaggatgaactctccaatcctgtcacttctggagaatcagtttccatctcctgcaggtctagtaagagtctcctatataaggatgggaagacatacttgaattggtttctgcagagaccaggacaatctcctcagctcctgatctatttgatgtccacccgtgcatccggagtctcagaccggtttagtggcagtgggtcaggaacagatttcaccctggaaatcagtagagtgaaggctgaggatgtgggtgtgtattactgtcaacaacttgtagagtatcctcgcacgttcggaggggggaccaagctggaaataaaa

SEQ ID NO: 103 - DNA, 366 bp, synthetic construct
  source 1..366: mol_type = other DNA
gaggtgaagctgcaggagtcaggccctgggatgttgcagccctcccagaccctcagtctgacttgttctttctctgggttttcactgagcacttctggtatgggtgtgagctggattcgtcagccttcaggaaagggtctggagtggctggcacacatttactgggatgatgacaaaaactttaatccatccctgaggagccgactcataatctccaaggacccctcccgaaaccaggttttcctcgagatcaccagtgtggacactgcggataccgccacatatttctgtgctcgaaaactctacaatgattacgactatattttggactactggggtcagggaacctcagtcaccgtctcctca

SEQ ID NO: 104 - DNA, 333 bp, synthetic construct; identical to SEQ ID NO: 100
  source 1..333: mol_type = other DNA

SEQ ID NO: 105 - DNA, 375 bp, synthetic construct
  source 1..375: mol_type = other DNA
caagtgaagctggaggagtcaggacctgaactggtgaaacctggggcctcagtgaagatttcctgcaaagcttctggctacgcattcagtagttcttgggtgaactgggtgcagcagaggcctggacagggtcttgagtggattggacggatttatcctggagatggagaaactaaatacagtggaaaatttaggggcaaggccacactgactgcagacaaatcctccaacacagtctatatgcaggtcagcagcctgacctctgtggactctgcggtctatttctgtgcaagagagggaggcctgattacgtcgagtgggtattaccatgctatggactactggggtcaaggaacctcagtcaccgtctcctca

SEQ ID NO: 106 - DNA, 330 bp, synthetic construct
  source 1..330: mol_type = other DNA
gacattgtgctcacacaatctccaccttctttggctgtgtctctaggtcagagggccaccatatcctgcagagccagtaaaagtgttgatagttatggcaatggttttatgcactggtaccagcagaaaccaggacagccacccaaactcctcatctttcttgcatccaacctagagtctggggtccctgccaggttcagtggcagtgggtctaggacagacttcaccctcaccattgatcctgtggaggctgatgatgctgcaagttattattgtcagcaaagtgatgaggatccgacgttcggcggaggcaccaagttggaaatcaaa

SEQ ID NO: 107 - DNA, 375 bp, synthetic construct
  source 1..375: mol_type = other DNA
caggttcagctggaggagtctggacctgagctggtgaagcctggggcctcagtgaagatttcctgcaaagcttctggctacgcattcagtagttcttggatgaactgggtgaagcagaggcctggacagggtcttgagtggattggacggatttatccaggagatggagatactcaataccatgggaaggtcaagggcaaggccacactgactgcagacaaatcctccagcacagcctacatgcaggtcagcagcctgacctctgtggactctgcggtctatttctgtgcaagagagggaggcatgattacgtcgaatggatactaccatgctttggactactggggtcaaggaacctcagtcaccgtctcctca

SEQ ID NO: 108 - DNA, 330 bp, synthetic construct
  source 1..330: mol_type = other DNA
gacattgtgatgacacagactacagcttctttggctgtgtctcaagggcagagggccaccatatcctgcagcgccagtgaaagtgttgatagttatggcaatagttttatgaactggtaccagcagaaaccaggacagccacccaaagtcctcatctatcttgcatccaacctagaatctggggtccctgccaggttcagtggcagtgggtctaggacagacttcaccctcaccattgatcctgtggaggctgatgatgctgcaacctattactgtcaacaaaataatgaggatccgacgttcggtggaggcaccaagctggaaatcaaa

SEQ ID NO: 109 - protein, 16 aa, synthetic construct
RSSKSLLHSNGITYLG

SEQ ID NO: 110 - protein, 16 aa, synthetic construct
RSSKSLLHSNGITYLI

SEQ ID NO: 111 - protein, 16 aa, synthetic construct
RSSKSLLHSNGITYLA

SEQ ID NO: 112 - protein, 16 aa, synthetic construct
RSSKSLLHSNGITYLM

SEQ ID NO: 113 - protein, 16 aa, synthetic construct
RSSKSLLHSNGITYLQ

SEQ ID NO: 114 - protein, 16 aa, synthetic construct
RSSKSLLHSNGITYLN

SEQ ID NO: 115 - protein, 16 aa, synthetic construct
RSSKSLLHSNGITYLV

SEQ ID NO: 116 - protein, 16 aa, synthetic construct
RSSKSLLHSNGITYLP

SEQ ID NO: 117 - protein, 330 aa, synthetic construct
ASTKGPSVFPLAPSSKSTSGGTAALGCLVKDYFPEPVTVSWNSGALTSGVHTFPAVLQSSGLYSLSSVVTVPSSSLGTQTYICNVNHKPSNTKVDKRVEPKSCDKTHTCPPCPAPELLGGPSVFLFPPKPKDTLYITREPEVTCVVVDVSHEDPEVKFNWYVDGVEVHNAKTKPREEQYNSTYRVVSVLTVLHQDWLNGKEYKCKVSNKALPAPIEKTISKAKGQPREPQVYTLPPSREEMTKNQVSLTCLVKGFYPSDIAVEWESNGQPENNYKTTPPVLDSDGSFFLYSKLTVDKSRWQQGNVFSCSVMHEALHNHYTQKSLSLSPGK

SEQ ID NO: 118 - protein, 107 aa, synthetic construct [sequence omitted]

SEQ ID NO: 119 - protein, 218 aa, synthetic construct
DIVMTQSPLSLPVTPGEPASISCRSSKSLLHSNGITYLCWFLQKPGQSPQLLIYQMSNLASGVPDRFSGSGSGTDFTLKISRVEAEDVGVYYCAQNLELWTFGQGTRLEIKRTVAAPSVFIFPPSDEQLKSGTASVVCLLNNFYPREAKVQWKVDNALQSGNSQESVTEQDSKDSTYSLSSTLTLSKADYEKHKVYACEVTHQGLSSPVTKSFNRGEC

SEQ ID NO: 120 - protein, 452 aa, synthetic construct
QVTLKESGPALVKPTQTLTLTCTFSGFSLSTSGMGVSWIRQPPGKALEWLAHIYWDDDKNFNPSLRSRLTITKDPSKNQVVLTMTNMDPVDTATYFCARKLYNDYDYILDYWGQGTTVTVSSASTKGPSVFPLAPSSKSTSGGTAALGCLVKDYFPEPVTVSWNSGALTSGVHTFPAVLQSSGLYSLSSVVTVPSSSLGTQTYICNVNHKPSNTKVDKRVEPKSCDKTHTCPPCPAPELLGGPSVFLFPPKPKDTLYITREPEVTCVVVDVSHEDPEVKFNWYVDGVEVHNAKTKPREEQYNSTYRVVSVLTVLHQDWLNGKEYKCKVSNKALPAPIEKTISKAKGQPREPQVYTLPPSREEMTKNQVSLTCLVKGFYPSDIAVEWESNGQPENNYKTTPPVLDSDGSFFLYSKLTVDKSRWQQGNVFSCSVMHEALHNHYTQKSLSLSPGK

SEQ ID NO: 121 - protein, 218 aa, synthetic construct
DIVMTQSPLSLPVTPGEPASISCRSSKSLLHSNGITYLGWFLQKPGQSPQLLIYQMSNLASGVPDRFSGSGSGTDFTLKISRVEAEDVGVYYCAQNLELWTFGQGTRLEIKRTVAAPSVFIFPPSDEQLKSGTASVVCLLNNFYPREAKVQWKVDNALQSGNSQESVTEQDSKDSTYSLSSTLTLSKADYEKHKVYACEVTHQGLSSPVTKSFNRGEC

SEQ ID NO: 122 - protein, 452 aa, synthetic construct; identical to SEQ ID NO: 120

SEQ ID NO: 123 - protein, 218 aa, synthetic construct
DIVMTQSPLSLPVTPGEPASISCRSSKSLLHSNGITYLAWFLQKPGQSPQLLIYQMSNLASGVPDRFSGSGSGTDFTLKISRVEAEDVGVYYCAQNLELWTFGQGTRLEIKRTVAAPSVFIFPPSDEQLKSGTASVVCLLNNFYPREAKVQWKVDNALQSGNSQESVTEQDSKDSTYSLSSTLTLSKADYEKHKVYACEVTHQGLSSPVTKSFNRGEC

SEQ ID NO: 124 - protein, 452 aa, synthetic construct; identical to SEQ ID NO: 120